European Patent Application EP 4 219 520 A1, published August 2, 2023. Title: METHOD FOR PRODUCING NUCLEIC ACID OLIGOMER. Applicant: SUMITOMO CHEMICAL COMPANY, LIMITED. The sequence listing filed with the application follows.

SEQUENCE LISTING (13 sequences)

SEQ ID NO: 1 - RNA, 24 nt, Artificial Sequence
  Synthetic oligonucleotide
agcagaguacacacagcauauacc

SEQ ID NO: 2 - RNA, 26 nt, Artificial Sequence
  Synthetic oligonucleotide
gguauaugcuguguguacucugcuuc

SEQ ID NO: 3 - RNA, 21 nt, Artificial Sequence
  Synthetic oligonucleotide
  modified_base (7)..(7), (17)..(17): um
  modified_base (19)..(20): thymidine(dT)
auggaanacucuuggunacnn

SEQ ID NO: 4 - RNA, 21 nt, Artificial Sequence
  Synthetic oligonucleotide
  modified_base (2)..(2), (12)..(12), (14)..(15), (19)..(19): um
  modified_base (5)..(6), (16)..(17): cm
  modified_base (20)..(21): thymidine(dT)
gnaannaagagnannnnannn

SEQ ID NO: 5 - DNA, 36 bp, Artificial Sequence
  Synthetic oligonucleotide
agagccagccuucuuauuguuuuagagcuaugcugu

SEQ ID NO: 6 - RNA, 23 nt, Artificial Sequence
  Synthetic oligonucleotide
ccaugagaaguaugacaacagcc

SEQ ID NO: 7 - RNA, 25 nt, Artificial Sequence
  Synthetic oligonucleotide
ggcuguugucauacuucucaugguu

SEQ ID NO: 8 - DNA, 67 bp, Artificial Sequence
  Synthetic oligonucleotide
acagcauagcaaguuaaaauaaggcuaguccguuaucaacuugaaaaaguggcaccgagucggugcu

SEQ ID NO: 9 - DNA, 94 bp, Artificial Sequence
  Synthetic oligonucleotide
guuuucccuuuucaaagaaaucuccugggcaccuaucuucuuaggugcccucccuuguuuaaaccugaccaguuaaccggcugguuagguuuuu

SEQ ID NO: 10 - DNA, 100 bp, Artificial Sequence
  Synthetic oligonucleotide
aguccucaucucccucaagcguuuuagagcuaguaauagcaaguuaaaauaaggcuaguccguuaucaacuugaaaaaguggcaccgagucggugcuuuu

SEQ ID NO: 11 - DNA, 113 bp, Artificial Sequence
  Synthetic oligonucleotide
gcagauguaguguuuccacaguuuaagagcuaugcuggaaacagcauagcaaguuuaaauaaggcuaguccguuaucaacuugaaaaaguggcaccgagucggugcuuuuuuu

SEQ ID NO: 12 - DNA, 113 bp, Artificial Sequence
  Synthetic oligonucleotide
  modified_base (1)..(1), (8)..(8), (17)..(18): thymidine(dT)
  modified_base (2)..(2), (19)..(19): 2'-deoxyguanosine
  modified_base (3)..(3), (6)..(6), (9)..(9), (11)..(11), (15)..(15): 2'-deoxythymidine
  modified_base (4)..(5), (7)..(7), (10)..(10), (12)..(14), (16)..(16), (20)..(20): 2'-deoxycytidine
nnnnnnnnnnnnnnnnnnnnguuuaagagcuaugcugguaacagcauagcaaguuuaaauaaggcuaguccguuaucaacuugaaaaaguggcaccgagucggugcuuuuuuu

SEQ ID NO: 13 - DNA, 113 bp, Artificial Sequence
  Synthetic oligonucleotide
  modified_base (1)..(1): phosphorothioate derivative of 2'-O-methyladenosine
  modified_base (2)..(2): phosphorothioate derivative of 2'-O-methylguanosine (gm)
  modified_base (3)..(3), (110)..(112): phosphorothioate derivative of 2'-O-methyluridine (um)
nnnccucaucucccucaagcguuuaagagcuaugcugguaacagcauagcaaguuuaaauaaggcuaguccguuaucaacuugaaaaaguggcaccgagucggugcuuunnnu